European Patent Application EP 4 596 568 A1, published August 6, 2025. Title: ペプチド合成方法. Applicant: 学校法人神戸学院. The sequence listing filed with the application follows.

SEQUENCE LISTING (6 sequences)

SEQ ID NO: 1 - protein, 5 aa, synthetic construct
YGGFL

SEQ ID NO: 2 - protein, 7 aa, synthetic construct
YAFGYPS

SEQ ID NO: 3 - protein, 5 aa, synthetic construct
YIGSR

SEQ ID NO: 4 - protein, 5 aa, synthetic construct
VAVAG

SEQ ID NO: 5 - protein, 8 aa, synthetic construct
CYIQNCPL

SEQ ID NO: 6 - protein, 31 aa, synthetic construct
TGGFMTSEKSQTPLVTLFKNAIIKNATKKGE